European Patent Specification EP 3 630 819 B1, published October 11, 2023. Title: DOSAGE AND ADMINISTRATION OF ANTI-C5 ANTIBODIES FOR TREATMENT OF PROTEIN-LOSING ENTEROPATHY IN PATIENTS. Applicant: ALEXION PHARMACEUTICALS, INC. The sequence listing filed with the application follows.

SEQUENCE LISTING (37 sequences)

SEQ ID NO: 1 - protein, 10 aa, Artificial Sequence
  source: /note="Description of Artificial Sequence: Synthetic peptide"
GYIFSNYWIQ

SEQ ID NO: 2 - protein, 17 aa, Artificial Sequence
  source: /note="Description of Artificial Sequence: Synthetic peptide"
EILPGSGSTEYTENFKD

SEQ ID NO: 3 - protein, 13 aa, Artificial Sequence
  source: /note="Description of Artificial Sequence: Synthetic peptide"
YFFGSSPNWYFDV

SEQ ID NO: 4 - protein, 11 aa, Artificial Sequence
  source: /note="Description of Artificial Sequence: Synthetic peptide"
GASENIYGALN

SEQ ID NO: 5 - protein, 7 aa, Artificial Sequence
  source: /note="Description of Artificial Sequence: Synthetic peptide"
GATNLAD

SEQ ID NO: 6 - protein, 9 aa, Artificial Sequence
  source: /note="Description of Artificial Sequence: Synthetic peptide"
QNVLNTPLT

SEQ ID NO: 7 - protein, 122 aa, Artificial Sequence [sequence omitted]

SEQ ID NO: 8 - protein, 107 aa, Artificial Sequence [sequence omitted]

SEQ ID NO: 9 - protein, 326 aa, Artificial Sequence
  source: /note="Description of Artificial Sequence: Synthetic polypeptide"
ASTKGPSVFPLAPCSRSTSESTAALGCLVKDYFPEPVTVSWNSGALTSGVHTFPAVLQSSGLYSLSSVVTVPSSNFGTQTYTCNVDHKPSNTKVDKTVERKCCVECPPCPAPPVAGPSVFLFPPKPKDTLMISRTPEVTCVVVDVSQEDPEVQFNWYVDGVEVHNAKTKPREEQFNSTYRVVSVLTVLHQDWLNGKEYKCKVSNKGLPSSIEKTISKAKGQPREPQVYTLPPSQEEMTKNQVSLTCLVKGFYPSDIAVEWESNGQPENNYKTTPPVLDSDGSFFLYSRLTVDKSRWQEGNVFSCSVMHEALHNHYTQKSLSLSLGK

SEQ ID NO: 10 - protein, 448 aa, Artificial Sequence
  source: /note="Description of Artificial Sequence: Synthetic polypeptide"
QVQLVQSGAEVKKPGASVKVSCKASGYIFSNYWIQWVRQAPGQGLEWMGEILPGSGSTEYTENFKDRVTMTRDTSTSTVYMELSSLRSEDTAVYYCARYFFGSSPNWYFDVWGQGTLVTVSSASTKGPSVFPLAPCSRSTSESTAALGCLVKDYFPEPVTVSWNSGALTSGVHTFPAVLQSSGLYSLSSVVTVPSSNFGTQTYTCNVDHKPSNTKVDKTVERKCCVECPPCPAPPVAGPSVFLFPPKPKDTLMISRTPEVTCVVVDVSQEDPEVQFNWYVDGVEVHNAKTKPREEQFNSTYRVVSVLTVLHQDWLNGKEYKCKVSNKGLPSSIEKTISKAKGQPREPQVYTLPPSQEEMTKNQVSLTCLVKGFYPSDIAVEWESNGQPENNYKTTPPVLDSDGSFFLYSRLTVDKSRWQEGNVFSCSVMHEALHNHYTQKSLSLSLGK

SEQ ID NO: 11 - protein, 214 aa, Artificial Sequence [sequence omitted]

SEQ ID NO: 12 - protein, 5 aa, Artificial Sequence
  source: /note="Description of Artificial Sequence: Synthetic peptide"
SYAIS

SEQ ID NO: 13 - protein, 17 aa, Artificial Sequence
  source: /note="Description of Artificial Sequence: Synthetic peptide"
GIGPFFGTANYAQKFQG

SEQ ID NO: 14 - protein, 7 aa, Artificial Sequence
  source: /note="Description of Artificial Sequence: Synthetic peptide"
DTPYFDY

SEQ ID NO: 15 - protein, 11 aa, Artificial Sequence
  source: /note="Description of Artificial Sequence: Synthetic peptide"
SGDSIPNYYVY

SEQ ID NO: 16 - protein, 7 aa, Artificial Sequence
  source: /note="Description of Artificial Sequence: Synthetic peptide"
DDSNRPS

SEQ ID NO: 17 - protein, 11 aa, Artificial Sequence
  source: /note="Description of Artificial Sequence: Synthetic peptide"
QSFDSSLNAEV

SEQ ID NO: 18 - protein, 116 aa, Artificial Sequence
  source: /note="Description of Artificial Sequence: Synthetic polypeptide"
QVQLVQSGAEVKKPGSSVKVSCKASGGTFSSYAISVWRQAPGQGLEWMGGIGPFFGTANYAQKFQGRVTITADESTSTAYMELSSLRSEDTAVYYCARDTPYFDYWGQGTLVTVSS

SEQ ID NO: 19 - protein, 108 aa, Artificial Sequence
  source: /note="Description of Artificial Sequence: Synthetic polypeptide"
DIELTQPPSVSVAPGQTARISCSGDSIPNYYVYWYQQKPGQAPVLVIYDDSNRPSGIPERFSGSNSGNTATLTISGTQAEDEADYYCQSFDSSLNAEVFGGGTKLTVL

SEQ ID NO: 20 - protein, 4 aa, Artificial Sequence
  source: /note="Description of Artificial Sequence: Synthetic peptide"
NYIS

SEQ ID NO: 21 - protein, 17 aa, Artificial Sequence
  source: /note="Description of Artificial Sequence: Synthetic peptide"
IIDPDDSYTEYSPSFQG

SEQ ID NO: 22 - protein, 8 aa, Artificial Sequence
  source: /note="Description of Artificial Sequence: Synthetic peptide"
YEYGGFDI

SEQ ID NO: 23 - protein, 11 aa, Artificial Sequence
  source: /note="Description of Artificial Sequence: Synthetic peptide"
SGDNIGNSYVH

SEQ ID NO: 24 - protein, 7 aa, Artificial Sequence
  source: /note="Description of Artificial Sequence: Synthetic peptide"
KDNDRPS

SEQ ID NO: 25 - protein, 9 aa, Artificial Sequence
  source: /note="Description of Artificial Sequence: Synthetic peptide"
GTYDIESYV

SEQ ID NO: 26 - protein, 116 aa, Artificial Sequence
  source: /note="Description of Artificial Sequence: Synthetic polypeptide"
EVQLVQSGAEVKKPGESLKISCKGSGYSFTNYISWVRQMPGKGLEWMGIIDPDDSYTEYSPSFQGQVTISADKSISTAYLQWSSLKASDTAMYYCARYEYGGFDIWGQGTLVTVSS

SEQ ID NO: 27 - protein, 106 aa, Artificial Sequence
  source: /note="Description of Artificial Sequence: Synthetic polypeptide"
SYELTQPPSVSVAPGQTARISCSGDNIGNSYVHWYQQKPGQAPVLVIYKDNDRPSGIPERFSGSNSGNTATLTISGTQAEDEADYYCGTYDIESYVFGGGTKLTVL

SEQ ID NO: 28 - protein, 6 aa, Artificial Sequence
  source: /note="Description of Artificial Sequence: Synthetic peptide"
SSYYVA

SEQ ID NO: 29 - protein, 17 aa, Artificial Sequence
  source: /note="Description of Artificial Sequence: Synthetic peptide"
AIYTGSGATYKASWAKG

SEQ ID NO: 30 - protein, 13 aa, Artificial Sequence
  source: /note="Description of Artificial Sequence: Synthetic peptide"
DGGYDYPTHAMHY

SEQ ID NO: 31 - protein, 11 aa, Artificial Sequence
  source: /note="Description of Artificial Sequence: Synthetic peptide"
QASQNIGSSLA

SEQ ID NO: 32 - protein, 7 aa, Artificial Sequence
  source: /note="Description of Artificial Sequence: Synthetic peptide"
GASKTHS

SEQ ID NO: 33 - protein, 12 aa, Artificial Sequence
  source: /note="Description of Artificial Sequence: Synthetic peptide"
QSTKVGSSYGNH

SEQ ID NO: 34 - protein, 123 aa, Artificial Sequence
  source: /note="Description of Artificial Sequence: Synthetic polypeptide"
QVQLVESGGGLVQPGGSLRLSCAASGFTSHSSYYVAWVRQAPGKGLEWVGAIYTGSGATYKASWAKGRFTISKDTSKNQVVLTMTNMDPVDTATYYCASDGGYDYPTHAMHYWGQGTLVTVSS

SEQ ID NO: 35 - protein, 110 aa, Artificial Sequence
  source: /note="Description of Artificial Sequence: Synthetic polypeptide"
DVVMTQSPSSLSASVGDRVTITCQASQNIGSSLAWYQQKPGQAPRLLIYGASKTHSGVPSRFSGSGSGTDFTLTISSLQPEDVATYYCQSTKVGSSYGNHFGGGTKVEIK

SEQ ID NO: 36 - DNA, 20 bp, Artificial Sequence
  source: /note="Description of Artificial Sequence: Synthetic primer"
acgaggcttctgcttactgc

SEQ ID NO: 37 - DNA, 20 bp, Artificial Sequence
  source: /note="Description of Artificial Sequence: Synthetic primer"
cagagaccgacttggacctc